European Patent Application EP 4 378 952 A1, published June 5, 2024. Title: UNIVERSAL T CELL AND APPLICATION THEREOF. Applicant: ST PHI THERAPEUTICS CO., LTD. Application EP. The sequence listing filed with the application follows.

SEQUENCE LISTING (131 sequences)

SEQ ID NO: 1 - protein, 144 aa, Homo sapiens
IWSAVFLNSLFNQEVQIPLTESYCGPCPKNWICYKNNCYQFFDESKNWYESQASCMSQNASLLKVYSKEDQDLLKLVKSYHWMGLVHIPTNGSWQWEDGSILSPNLLTIIEMQKGDCALYASSFKGYIENCSTPNTYICMQRTV

SEQ ID NO: 2 - protein, 216 aa, Homo sapiens
MGWIRGRRSRHSWEMSEFHNYNLDLKKSDFSTRWQKQRCPVVKSKCRENASPFFFCCFIAVAMGIRFIIMVTIWSAVFLNSLFNQEVQIPLTESYCGPCPKNWICYKNNCYQFFDESKNWYESQASCMSQNASLLKVYSKEDQDLLKLVKSYHWMGLVHIPTNGSWQWEDGSILSPNLLTIIEMQKGDCALYASSFKGYIENCSTPNTYICMQRTV

SEQ ID NO: 3 - protein, 143 aa, Mus musculus
FKETFQPVLCNKEVPVSSREGYCGPCPNNWICHRNNCYQFFNEEKTWNQSQASCLSQNSSLLKIYSKEEQDFLKLVKSYHWMGLVQIPANGSWQWEDGSSLSYNQLTLVEIPKGSCAVYGSSFKAYTEDCANLNTYICMKRAV

SEQ ID NO: 4 - protein, 232 aa, Mus musculus
MALIRDRKSHHSEMSKCHNYDLKPAKWDTSQEQQKQRLALTTSQPGENGIIRGRYPIEKLKISPMFVVRVLAIALAIRFTLNTLMWLAIFKETFQPVLCNKEVPVSSREGYCGPCPNNWICHRNNCYQFFNEEKTWNQSQASCLSQNSSLLKIYSKEEQDFLKLVKSYHWMGLVQIPANGSWQWEDGSSLSYNQLTLVEIPKGSCAVYGSSFKAYTEDCANLNTYICMKRAV

SEQ ID NO: 5 - protein, 220 aa, synthetic construct
MGWIRGRRSRHSWEMSEFHNYNLDLKKSDFSTRWQKQRCPVVKSKCRENASPMFVVRVLAIALAIRFTLNTLMWLAIFKETFQPVLFNQEVQIPLTESYCGPCPKNWICYKNNCYQFFDESKNWYESQASCMSQNASLLKVYSKEDQDLLKLVKSYHWMGLVHIPTNGSWQWEDGSILSPNLLTIIEMQKGDCALYASSFKGYIENCSTPNTYICMQRTV

SEQ ID NO: 6 - protein, 231 aa, Homo sapiens
MSKQRGTFSEVSLAQDPKRQQRKPKGNKSSISGTEQEIFQVELNLQNPSLNHQGIDKIYDCQGLLPPPEKLTAEVLGIICIVLMATVLKTIVLIPFLEQNNSSPNTRTQKARHCGHCPEEWITYSNSCYYIGKERRTWEESLLACTSKNSSLLSIDNEEEMKFLASILPSSWIGVFRNSSHHPWVTINGLAFKHKIKDSDNAELNCAVLQVNRLKSAQCGSSMIYHCKHKL

SEQ ID NO: 7 - protein, 240 aa, Homo sapiens
MSKQRGTFSEVSLAQDPKWQQRKPKGNKSSISGTEQEIFQVELNLQNASLNHQGIDKIYDCQGLLPPPEKLTAEVLGIICIVLMATVLKTIVLIPFLEQNNSSPNARTQKARHCGHCPEEWITYSNSCYYIGKERRTWEESLQACASKNSSSLLCIDNEEEMKFLASILPSSWIGVFRNSSHHPWVTINGLAFKHEIKDSDHAERNCAMLHVRGLISDQCGSSRIIRRGFIMLTRLVLNS

SEQ ID NO: 8 - protein, 158 aa, Homo sapiens
MNKQRGTYSEVSLAQDPKRQQRKLKGNKISISGTKQEIFQVELNLQNASSDHQGNDKTYHCKGLLPPPEKLTAEVLGIICIVLMATVLKTIVLIPCIGVLEQNNFSLNRRMQKARHCGHCPEEWITYSNSCYYIGKERRTWEERVCWPVLRRTLICFL

SEQ ID NO: 9 - protein, 179 aa, Homo sapiens
MAVFKTTLWRLISGTLGIICLSLMSTLGILLKNSFTKLSIEPAFTPGPNIELQKDSDCCSCQEKWVGYRCNCYFISSEQKTWNESRHLCASQKSSLLQLQNTDELDFMSSSQQFYWIGLSYSEEHTAWLWENGSALSQYLFPSFETFNTKNCIAYNPNGNALDESCEDKNRYICKQQLI

SEQ ID NO: 10 - protein, 377 aa, Homo sapiens
MSMSPTVIILACLGFFLDQSVWAHVGGQDKPFCSAWPSAVVPQGGHVTLRCHYRRGFNIFTLYKKDGVPVPELYNRIFWNSFLISPVTPAHAGTYRCRGFHPHSPTEWSAPSNPLVIMVTGLYEKPSLTARPGPTVRAGENVTLSCSSQSSFDIYHLSREGEAHELRLPAVPSINGTFQADFPLGPATHGETYRCFGSFHGSPYEWSDPSDPLPVSVTGNPSSSWPSPTEPSFKTGIARHLHAVIRYSVAIILFTILPFFLLHRWCSKKKDAAVMNQEPAGHRTVNREDSDEQDPQEVTYAQLDHCIFTQRKITGPSQRSKRPSTDTSVCIELPNAEPRALSPAHEHHSQALMGSSRETTALSQTQLASSNVPAAGI

SEQ ID NO: 11 - protein, 304 aa, Homo sapiens
MSLTVVSMACVGFFLLQGAWPHEGVHRKPSLLAHPGRLVKSEETVILQCWSDVMFEHFLLHREGMFNDTLRLIGEHHDGVSKANFSISRMKQDLAGTYRCYGSVTHSPYQLSAPSDPLDIVIIGLYEKPSLSAQPGPTVLAGENVTLSCSSRSSYDMYHLSREGEAHERRLPAGTKVNGTFQANFPLGPATHGGTYRCFGSFRDSPYEWSKSSDPLLVSVTGNPSNSWPSPTEPSSETGNPRHLHVLIGTSVVKIPFTILLFFLLHRWCSDKKNAAVMDQEPAGNRTVNSEDSDEQDHQEVSYA

SEQ ID NO: 12 - protein, 304 aa, Homo sapiens
MSLMVVSMACVGFFLLQGAWPHEGVHRKPSLLAHPGPLVKSEETVILQCWSDVRFEHFLLHREGKYKDTLHLIGEHHDGVSKANFSIGPMMQDLAGTYRCYGSVTHSPYQLSAPSDPLDIVITGLYEKPSLSAQPGPTVLAGESVTLSCSSRSSYDMYHLSREGEAHERRFSAGPKVNGTFQADFPLGPATHGGTYRCFGSFRDSPYEWSNSSDPLLVSVTGNPSNSWPSPTEPSSKTGNPRHLHVLIGTSVVKIPFTILLFFLLHRWCSNKKNAAVMDQEPAGNRTVNSEDSDEQDHQEVSYA

SEQ ID NO: 13 - protein, 304 aa, Homo sapiens
MSLMVIIMACVGFFLLQGAWPQEGVHRKPSFLALPGHLVKSEETVILQCWSDVMFEHFLLHREGKFNNTLHLIGEHHDGVSKANFSIGPMMPVLAGTYRCYGSVPHSPYQLSAPSDPLDMVIIGLYEKPSLSAQPGPTVQAGENVTLSCSSRSSYDMYHLSREGEAHERRLPAVRSINGTFQADFPLGPATHGGTYRCFGSFRDAPYEWSNSSDPLLVSVTGNPSNSWPSPTEPSSKTGNPRHLHVLIGTSVVKIPFTILLFFLLHRWCSDKKNAAVMDQEPAGNRTVNSEDSDEQDHQEVSYA

SEQ ID NO: 14 - protein, 382 aa, Homo sapiens
MLLMVVSMACVGLFLVQRAGPHMGGQDKPFLSAWPSAVVPRGGHVTLRCHYRHRFNNFMLYKEDRIHVPIFHGRIFQEGFNMSPVTTAHAGNYTCRGSHPHSPTGWSAPSNPMVIMVTGNHRKPSLLAHPGPLVKSGERVILQCWSDIMFEHFFLHREWISKDPSRLVGQIHDGVSKANFSIGSMMRALAGTYRCYGSVTHTPYQLSAPSDPLDIVVTGLYEKPSLSAQPGPKVQAGESVTLSCSSRSSYDMYHLSREGGAHERRLPAVRKVNRTFQADFPLGPATHGGTYRCFGSFRHSPYEWSDPSDPLLVSVTGNPSSSWPSPTEPSSKSGNLRHLHILIGTSVVKIPFTILLFFLLHRWCSNKKKCCCNGPRACREQK

SEQ ID NO: 15 - protein, 304 aa, Homo sapiens
MSSTLPALLCVGLCLSQRISAQQQTLPKPFIWAEPHFMVPKEKQVTICCQGNYGAVEYQLHFEGSLFAVDRPKPPERINKVKFYIPDMNSRMAGQYSCIYRVGELWSEPSNLLDLVVTEMYDTPTLSVHPGPEVISGEKVTFYCRLDTATSMFLLLKEGRSSHVQRGYGKVQAEFPLGPVTTAHRGTYRCFGSYNNHAWSFPSEPVKLLVTGDIENTSLAPEDPTFPADTWGTYLLTTETGLQKDHALWDHTAQNLLRMGLAFLVLVALVWFLVEDWLSRKRTRERASRASTWEGRRRLNTQTL

SEQ ID NO: 16 - protein, 276 aa, Homo sapiens
MAWRALHPLLLLLLLFPGSQAQSKAQVLQSVAGQTLTVRCQYPPTGSLYEKKGWCKEASALVCIRLVTSSKPRTMAWTSRFTIWDDPDAGFFTVTMTDLREEDSGHYWCRIYRPSDNSVSKSVRFYLVVSPASASTQTSWTPRDLVSSQTQTQSCVPPTAGARQAPESPSTIPVPSQPQNSTLRPGPAAPIALVPVFCGLLVAKSLVLSALLVWWGDIWWKTMMELRSLDTQKATCHLQQVTDLPWTSVSSPVEREILYHTVARTKISDDDDEHTL

SEQ ID NO: 17 - protein, 201 aa, Homo sapiens
MAWMLLLILIMVHPGSCALWVSQPPEIRTLEGSSAFLPCSFNASQGRLAIGSVTWFRDEVVPGKEVRNGTPEFRGRLAPLASSRFLHDHQAELHIRDVRGHDASIYVCRVEVLGLGVGTGNGTRLVVEKEHPQLGAGTVLLLRAGFYAVSFLSVAVGSTVYYQGKCLTWKGPRRQLPAVVPAPLPPPCGSSAHLLPPVPGG

SEQ ID NO: 18 - protein, 336 aa, Homo sapiens
MDYPTLLLALLHVYRALCEEVLWHTSVPFAENMSLECVYPSMGILTQVEWFKIGTQQDSIAIFSPTHGMVIRKPYAERVYFLNSTMASNNMTLFFRNASEDDVGYYSCSLYTYPQGTWQKVIQVVQSDSFEAAVPSNSHIVSEPGKNVTLTCQPQMTWPVQAVRWEKIQPRQIDLLTYCNLVHGRNFTSKFPRQIVSNCSHGRWSVIVIPDVTVSDSGLYRCYLQASAGENETFVMRLTVAEGKTDNQYTLFVAGGTVLLLLFVISITTIIVIFLNRRRRRERRDLFTESWDTQKAPNNYRSPISTSQPTNQSMDDTREDIYVNYPTFSRRPKTRV

SEQ ID NO: 19 - protein, 281 aa, Homo sapiens [sequence omitted]

SEQ ID NO: 20 - protein, 254 aa, Homo sapiens
MWQLLLPTALLLLVSAGMRTEDLPKAVVFLEPQWYRVLEKDSVTLKCQGAYSPEDNSTQWFHNESLISSQASSYFIDAATVDDSGEYRCQTNLSTLSDPVQLEVHIGWLLLQAPRWVFKEEDPIHLRCHSWKNTALHKVTYLQNGKGRKYFHHNSDFYIPKATLKDSGSYFCRGLFGSKNVSSETVNITITQGLAVSTISSFFPPGYQVSFCLVMVLLFAVDTGLYFSVKTNIRSSTRDWKDHKFKWRKDPQDK

SEQ ID NO: 21 - protein, 370 aa, Homo sapiens
MLGQVVTLILLLLLKVYQGKGCQGSADHVVSISGVPLQLQPNSIQTKVDSIAWKKLLPSQNGFHHILKWENGSLPSNTSNDRFSFIVKNLSLLIKAAQQQDSGLYCLEVTSISGKVQTATFQVFVFESLLPDKVEKPRLQGQGKILDRGRCQVALSCLVSRDGNVSYAWYRGSKLIQTAGNLTYLDEEVDINGTHTYTCNVSNPVSWESHTLNLTQDCQNAHQEFRFWPFLVIIVILSALFLGTLACFCVWRRKRKEKQSETSPKEFLTIYEDVKDLKTRRNHEQEQTFPGGGSTIYSMIQSQSSAPTSQEPAYTLYSLIQPSRKSGSRKRNHSPSFNSTIYEVIGKSQPKAQNPARLSRKELENFDVYS

SEQ ID NO: 22 - protein, 332 aa, Homo sapiens
MLWLFQSLLFVFCFGPGNVVSQSSLTPLMVNGILGESVTLPLEFPAGEKVNFITWLFNETSLAFIVPHETKSPEIHVTNPKQGKRLNFTQSYSLQLSNLKMEDTGSYRAQISTKTSAKLSSYTLRILRQLRNIQVTNHSQLFQNMTCELHLTCSVEDADDNVSFRWEALGNTLSSQPNLTVSWDPRISSEQDYTCIAENAVSNLSFSVSAQKLCEDVKIQYTDTKMILFMVSGICIVFGFIILLLLVLRKRRDSLSLSTQRTQGPAESARNLEYVSVSPTNNTVYASVTHSNRETEIWTPRENDTITIYSTINHSKESKPTFSRATALDNVV

SEQ ID NO: 23 - protein, 335 aa, Homo sapiens
MAGSPTCLTLIYILWQLTGSAASGPVKELVGSVGGAVTFPLKSKVKQVDSIVWTFNTTPLVTIQPEGGTIIVTQNRNRERVDFPDGGYSLKLSKLKKNDSGIYYVGIYSSSLQQPSTQEYVLHVYEHLSKPKVTMGLQSNKNGTCVTNLTCCMEHGEEDVIYTWKALGQAANESHNGSILPISWRWGESDMTFICVARNPVSRNFSSPILARKLCEGAADDPDSSMVLLCLLLVPLLLSLFVLGLFLWFLKRERQEEYIEEKKRVDICRETPNICPHSGENTEYDTIPHTNRTILKEDPANTVYSTVEIPKKMENPHSLLTMPDTPRLFAYENVI

SEQ ID NO: 24 - protein, 231 aa, Homo sapiens
MQDEERYMTLNVQSKKRSSAQTSQLTFKDYSVTLHWYKILLGISGTVNGILTLTLISLILLVSQGVLLKCQKGSCSNATQYEDTGDLKVNNGTRRNISNKDLCASRSADQTVLCQSEWLKYQGKCYWFSNEMKSWSDSYVYCLERKSHLLIIHDQLEMAFIQKNLRQLNYVWIGLNFTSLKMTWTWVDGSPIDSKIFFIKGPAKENSCAAIKESKIFSETCSSVFKWICQY

SEQ ID NO: 25 - protein, 93 aa, Homo sapiens
MIHLGHILFLLLLPVAAAQTTPGERSSLPAFYPGTSGSCSGCGSLSLPLLAGLVAADAVASLLIVGAVFLCARPRRSPAQEDGKVYINMPGRG

SEQ ID NO: 26 - protein, 92 aa, Homo sapiens
MIHLGHILFLLLLPVAAAQTTPGERSSLPAFYPGTSGSCSGCGSLSLPLLAGLVAADAVASLLIVGAVFLCARPRRSPAQDGKVYINMPGRG

SEQ ID NO: 27 - protein, 21 aa, Homo sapiens
LLAGLVAADAVASLLIVGAVF

SEQ ID NO: 28 - protein, 113 aa, Homo sapiens
MGGLEPCSRLLLLPLLLAVSGLRPVQAQAQSDCSCSTVSPGVLAGIVMGDLVLTVLIALAVYFLGRLVPRGRGAAEAATRKQRITETESPYQELQGQRSDVYSDLNTQRPYYK

SEQ ID NO: 29 - protein, 21 aa, Homo sapiens
GVLAGIVMGDLVLTVLIALAV

SEQ ID NO: 30 - protein, 38 aa, synthetic construct
GVLAGIVMGDLVLTVLIALAVLVAADAVASLLIVGAVF

SEQ ID NO: 31 - protein, 150 aa, synthetic construct
MIHLGHILFLLLLPVAAAQTTPGERSSLPAFYPGTSGSCSGCGSLSLPLLAGLVAADAVASLLIVGAVFLCARPRRSPAQEDGKVYINMPGRGGGGGSYFLGRLVPRGRGAAEAATRKQRITETESPYQELQGQRSDVYSDLNTQRPYYK

SEQ ID NO: 32 - protein, 112 aa, Homo sapiens
RVKFSRSADAPAYQQGQNQLYNELNLGRREEYDVLDKRRGRDPEMGGKPRRKNPQEGLYNELQKDKMAEAYSEIGMKGERRRGKGHDGLYQGLSTATKDTYDALHMQALPPR

SEQ ID NO: 33 - protein, 210 aa, synthetic construct
MIHLGHILFLLLLPVAAAQTTPGERSSLPAFYPGTSGSCSGCGSLSLPLLAGLVAADAVASLLIVGAVFLCARPRRSPAQEDGKVYINMPGRGGGGGSRVKFSRSADAPAYQQGQNQLYNELNLGRREEYDVLDKRRGRDPEMGGKPRRKNPQEGLYNELQKDKMAEAYSEIGMKGERRRGKGHDGLYQGLSTATKDTYDALHMQALPPR

SEQ ID NO: 34 - protein, 230 aa, synthetic construct
MGGLEPCSRLLLLPLLLAVSGLRPVQAQAQSDCSCSTVSPGVLAGIVMGDLVLTVLIALAVYFLGRLVPRGRGAAEAATRKQRITETESPYQELQGQRSDVYSDLNTQRPYYKGGGGSRVKFSRSADAPAYQQGQNQLYNELNLGRREEYDVLDKRRGRDPEMGGKPRRKNPQEGLYNELQKDKMAEAYSEIGMKGERRRGKGHDGLYQGLSTATKDTYDALHMQALPPR

SEQ ID NO: 35 - protein, 267 aa, synthetic construct
MIHLGHILFLLLLPVAAAQTTPGERSSLPAFYPGTSGSCSGCGSLSLPLLAGLVAADAVASLLIVGAVFLCARPRRSPAQEDGKVYINMPGRGGGGGSYFLGRLVPRGRGAAEAATRKQRITETESPYQELQGQRSDVYSDLNTQRPYYKGGGGSRVKFSRSADAPAYQQGQNQLYNELNLGRREEYDVLDKRRGRDPEMGGKPRRKNPQEGLYNELQKDKMAEAYSEIGMKGERRRGKGHDGLYQGLSTATKDTYDALHMQALPPR

SEQ ID NO: 36 - protein, 42 aa, Homo sapiens
KRGRKKLLYIFKQPFMRPVQTTQEEDGCSCRFPEEEEGGCEL

SEQ ID NO: 37 - protein, 140 aa, synthetic construct
MIHLGHILFLLLLPVAAAQTTPGERSSLPAFYPGTSGSCSGCGSLSLPLLAGLVAADAVASLLIVGAVFLCARPRRSPAQEDGKVYINMPGRGGGGGSKRGRKKLLYIFKQPFMRPVQTTQEEDGCSCRFPEEEEGGCEL

SEQ ID NO: 38 - protein, 252 aa, synthetic construct
MIHLGHILFLLLLPVAAAQTTPGERSSLPAFYPGTSGSCSGCGSLSLPLLAGLVAADAVASLLIVGAVFLCARPRRSPAQEDGKVYINMPGRGGGGGSKRGRKKLLYIFKQPFMRPVQTTQEEDGCSCRFPEEEEGGCELRVKFSRSADAPAYQQGQNQLYNELNLGRREEYDVLDKRRGRDPEMGGKPRRKNPQEGLYNELQKDKMAEAYSEIGMKGERRRGKGHDGLYQGLSTATKDTYDALHMQALPPR

SEQ ID NO: 39 - protein, 41 aa, Homo sapiens
RSKRSRLLHSDYMNMTPRRPGPTRKHYQPYAPPRDFAAYRS

SEQ ID NO: 40 - protein, 139 aa, synthetic construct
MIHLGHILFLLLLPVAAAQTTPGERSSLPAFYPGTSGSCSGCGSLSLPLLAGLVAADAVASLLIVGAVFLCARPRRSPAQEDGKVYINMPGRGGGGGSRSKRSRLLHSDYMNMTPRRPGPTRKHYQPYAPPRDFAAYRS

SEQ ID NO: 41 - protein, 251 aa, synthetic construct
MIHLGHILFLLLLPVAAAQTTPGERSSLPAFYPGTSGSCSGCGSLSLPLLAGLVAADAVASLLIVGAVFLCARPRRSPAQEDGKVYINMPGRGGGGGSRSKRSRLLHSDYMNMTPRRPGPTRKHYQPYAPPRDFAAYRSRVKFSRSADAPAYQQGQNQLYNELNLGRREEYDVLDKRRGRDPEMGGKPRRKNPQEGLYNELQKDKMAEAYSEIGMKGERRRGKGHDGLYQGLSTATKDTYDALHMQALPPR

SEQ ID NO: 42 - protein, 160 aa, synthetic construct
MGGLEPCSRLLLLPLLLAVSGLRPVQAQAQSDCSCSTVSPGVLAGIVMGDLVLTVLIALAVYFLGRLVPRGRGAAEAATRKQRITETESPYQELQGQRSDVYSDLNTQRPYYKGGGGSKRGRKKLLYIFKQPFMRPVQTTQEEDGCSCRFPEEEEGGCEL

SEQ ID NO: 43 - protein, 272 aa, synthetic construct
MGGLEPCSRLLLLPLLLAVSGLRPVQAQAQSDCSCSTVSPGVLAGIVMGDLVLTVLIALAVYFLGRLVPRGRGAAEAATRKQRITETESPYQELQGQRSDVYSDLNTQRPYYKGGGGSKRGRKKLLYIFKQPFMRPVQTTQEEDGCSCRFPEEEEGGCELRVKFSRSADAPAYQQGQNQLYNELNLGRREEYDVLDKRRGRDPEMGGKPRRKNPQEGLYNELQKDKMAEAYSEIGMKGERRRGKGHDGLYQGLSTATKDTYDALHMQALPPR

SEQ ID NO: 44 - protein, 159 aa, synthetic construct
MGGLEPCSRLLLLPLLLAVSGLRPVQAQAQSDCSCSTVSPGVLAGIVMGDLVLTVLIALAVYFLGRLVPRGRGAAEAATRKQRITETESPYQELQGQRSDVYSDLNTQRPYYKGGGGSRSKRSRLLHSDYMNMTPRRPGPTRKHYQPYAPPRDFAAYRS

SEQ ID NO: 45 - protein, 271 aa, synthetic construct
MGGLEPCSRLLLLPLLLAVSGLRPVQAQAQSDCSCSTVSPGVLAGIVMGDLVLTVLIALAVYFLGRLVPRGRGAAEAATRKQRITETESPYQELQGQRSDVYSDLNTQRPYYKGGGGSRSKRSRLLHSDYMNMTPRRPGPTRKHYQPYAPPRDFAAYRSRVKFSRSADAPAYQQGQNQLYNELNLGRREEYDVLDKRRGRDPEMGGKPRRKNPQEGLYNELQKDKMAEAYSEIGMKGERRRGKGHDGLYQGLSTATKDTYDALHMQALPPR

SEQ ID NO: 46 - protein, 199 aa, Human cytomegalovirus
MNNLWKAWVGLWTSMGPLIRLPDGITKAGEDALRPWKSTAKHPWFEIEDNRCYIDNGKLFARGSIVGNMSRFVFDPKADYGGVGENLYVHADDVEFVPGESLKWNVRNLDVMPIFETLALRLVLQGDVIWLRCVPELRVDYTSSAYMWNMQYGMVRKSYTHVAWTIVFYSINITLLVLFIVYVTVDCNLSMMWMRFFVC

SEQ ID NO: 47 - protein, 161 aa, Human cytomegalovirus
MNNLWKAWVGLWTSMGPLIRLPDGITKAGEDALRPWKSTAKHPWFEIEDNRCYIDNGKLFARGSIVGNMSRFVFDPKADYGGVGENLYVHADDVEFVPGESLKWNVRNLDVMPIFETLALRLVLQGDVIWLRCVPELRVDYTSSAYMWNMQYGMVRKSYTH

SEQ ID NO: 48 - protein, 38 aa, Human cytomegalovirus
VAWTIVFYSINITLLVLFIVYVTVDCNLSMMWMRFFVC

SEQ ID NO: 49 - protein, 186 aa, Human cytomegalovirus
MKPVLVLAILAVLFLRLADSVPRPLDVVVSEIRSAHFRVEENQCWFHMGMLYFKGRMSGNFTEKHFVNVGIVSQSYMDRLQVSGEQYHHDERGAYFEWNIGGHPVTHTVDMVDITLSTRWGDPKKYAACVPQVRMDYSSQTINWYLQRSMRDDNWGLLFRTLLVYLFSLVVLVLLTVGVSARLRFI

SEQ ID NO: 50 - protein, 160 aa, Human cytomegalovirus
MKPVLVLAILAVLFLRLADSVPRPLDVVVSEIRSAHFRVEENQCWFHMGMLYFKGRMSGNFTEKHFVNVGIVSQSYMDRLQVSGEQYHHDERGAYFEWNIGGHPVTHTVDMVDITLSTRWGDPKKYAACVPQVRMDYSSQTINWYLQRSMRDDNWGLLFR

SEQ ID NO: 51 - protein, 26 aa, Human cytomegalovirus
TLLVYLFSLVVLVLLTVGVSARLRFI

SEQ ID NO: 52 - protein, 215 aa, Human cytomegalovirus
MNLVMLILALWAPVAGSMPELSLTLFDEPPPLVETEPLPPLSDVSEYRVEYSEARCVLRSGGRLEALWTLRGNLSVPTPTPRVYYQTLEGYADRVPTPVEDVSESLVAKRYWLRDYRVPQRTKLVLFYFSPCHQCQTYYVECEPRCLVPWVPLWSSLEDIERLLFEDRRLMAYYALTIKSAQYTLMMVAVIQVFWGLYVKGWLHRHFPWMFSDQW

SEQ ID NO: 53 - protein, 165 aa, Human cytomegalovirus
MPELSLTLFDEPPPLVETEPLPPLSDVSEYRVEYSEARCVLRSGGRLEALWTLRGNLSVPTPTPRVYYQTLEGYADRVPTPVEDVSESLVAKRYWLRDYRVPQRTKLVLFYFSPCHQCQTYYVECEPRCLVPWVPLWSSLEDIERLLFEDRRLMAYYALTIKSAQ

SEQ ID NO: 54 - protein, 33 aa, Human cytomegalovirus
YTLMMVAVIQVFWGLYVKGWLHRHFPWMFSDQW

SEQ ID NO: 55 - protein, 185 aa, Human cytomegalovirus
MLRRGSLRNPLAICLLWWLGVVAAATEETREPTYFTCGCVIQNHVLKGAVKLYGQFPSPKTLRASAWLHDGENHERHRQPILVEGTATATEALYILLPTELSSPEGNRPRNYSATLTLASRDCYERFVCPVYDSGTPMGVLMNLTYLWYLGDYGAILKIYFGLFCGACVITRSLLLICGYYPPRE

SEQ ID NO: 56 - protein, 124 aa, Human cytomegalovirus
ATEETREPTYFTCGCVIQNHVLKGAVKLYGQFPSPKTLRASAWLHDGENHERHRQPILVEGTATATEALYILLPTELSSPEGNRPRNYSATLTLASRDCYERFVCPVYDSGTPMGVLMNLTYLW

SEQ ID NO: 57 - protein, 36 aa, Human cytomegalovirus
LGDYGAILKIYFGLFCGACVITRSLLLICGYYPPRE

SEQ ID NO: 58 - protein, 159 aa, Adenovirus type 37
MRYMILGLLALAAVCSAAKKVEFKEPACNVTFKSEANECTTLIKCTTEHEKLIIRHKDKIGKYAVYAIWQPGDTNDYNVTVFQGENRKTFMYKFPFYEMCDITMYMSKQYKLWPPQKCLENTGTFCSTALLITALALVCTLLYLKYKSRRSFIDEKKMP

SEQ ID NO: 59 - protein, 106 aa, Adenovirus type 37
AKKVEFKEPACNVTFKSEANECTTLIKCTTEHEKLIIRHKDKIGKYAVYAIWQPGDTNDYNVTVFQGENRKTFMYKFPFYEMCDITMYMSKQYKLWPPQKCLENTG

SEQ ID NO: 60 - protein, 36 aa, Adenovirus type 37
TFCSTALLITALALVCTLLYLKYKSRRSFIDEKKMP

SEQ ID NO: 61 - protein, 430 aa, Human herpesvirus 7
MWTILLFCVPVIYGELYPDFCPLAVVDFDVNATVDDLLLFDISLSKQCSDDKIRHSAVAAMTDNAFFFGNSETQIETDFGKYLAFNCYQVFSTLNHFLFKNFKKTKGLMKRYDKLCLDVESYIHIQIICSPFKSFIRLRRMNETGISPRILETTFYLQNKRNSTWVAIKNYLGEDDPFTYRIWHTLTHAKNFLINSCENDFNQLFFWQRKYLSLAKTFEATFKQGFNPMIEQRNEQRYRTNNIDCSFSKFRQNGVKVAVCKYTGWGVSGFGSLEVLQKIKSPFGEEWKRVGFNSTGAFTPLYGSDVLWGLIFLRVEMTTYVCTCTNKNTGTQIQVTLPDVDLDLLDSEKTSSNVFVDMLCYTLIAILFLAFVTAVVLLGVSCLDGVQKVLTWPLQHIQKEPVSEKIINLTNLMFGQEPLPKKESLKQQCL

SEQ ID NO: 62 - protein, 362 aa, Human herpesvirus 7
MWTILLFCVPVIYGELYPDFCPLAVVDFDVNATVDDLLLFDISLSKQCSDDKIRHSAVAAMTDNAFFFGNSETQIETDFGKYLAFNCYQVFSTLNHFLFKNFKKTKGLMKRYDKLCLDVESYIHIQIICSPFKSFIRLRRMNETGISPRILETTFYLQNKRNSTWVAIKNYLGEDDPFTYRIWHTLTHAKNFLINSCENDFNQLFFWQRKYLSLAKTFEATFKQGFNPMIEQRNEQRYRTNNIDCSFSKFRQNGVKVAVCKYTGWGVSGFGSLEVLQKIKSPFGEEWKRVGFNSTGAFTPLYGSDVLWGLIFLRVEMTTYVCTCTNKNTGTQIQVTLPDVDLDLLDSEKTSSNVFVDMLCYT

SEQ ID NO: 63 - protein, 68 aa, Human herpesvirus 7
LIAILFLAFVTAVVLLGVSCLDGVQKVLTWPLQHIQKEPVSEKIINLTNLMFGQEPLPKKESLKQQCL

SEQ ID NO: 64 - protein, 183 aa, Human cytomegalovirus
MDLLIRLGFLLMCALPTPGERSSRDPKTLLSLSPRQQACVPRTKSHRPVCYNDTGDCTDADDSWKQLGEDFAHQCLQAAKKRPKTHKSRPNDRNLEGRLTCQRVRRLLPCDLDIHPSHRLLTLMNNCVCDGAVWNAFRLIERHGFFAVTLYLCCGITLLVVILALLCSITYESTGRGIRRCGS

SEQ ID NO: 65 - protein, 125 aa, Human cytomegalovirus
ERSSRDPKTLLSLSPRQQACVPRTKSHRPVCYNDTGDCTDADDSWKQLGEDFAHQCLQAAKKRPKTHKSRPNDRNLEGRLTCQRVRRLLPCDLDIHPSHRLLTLMNNCVCDGAVWNAFRLIERHG

SEQ ID NO: 66 - protein, 88 aa, herpes simplex virus 7
MSWALEMADTFLDTMRVGPRTYADVRDEINKRGREDREAARTAVHDPERPLLRSPGLLPEIAPNASLGVAHRRTGGTVTDSPRNPVTR

SEQ ID NO: 67 - protein, 57 aa, herpes simplex virus 7
MSWALEMADTFLDTMRVGPRTYADVRDEINKRGREDREAARTAVHDPERPLLRSPGL

SEQ ID NO: 68 - protein, 160 aa, Cowpox virus
MFIMRELVYRVVIVILSLSLLSSFLVICFIEHRCFKEETRYKICPKNTISINNICYYFSEDTTNWTASFEYCKNMNGRLACIINDTFPKICRYKGTFDYWVGLYRTNSQSPWLNCDNKPYNNIIPIRGVEDYAYLNNNGISTARIYADRRWICEVPMVDY

SEQ ID NO: 69 - protein, 133 aa, Cowpox virus
CFIEHRCFKEETRYKICPKNTISINNICYYFSEDTTNWTASFEYCKNMNGRLACIINDTFPKICRYKGTFDYWVGLYRTNSQSPWLNCDNKPYNNIIPIRGVEDYAYLNNNGISTARIYADRRWICEVPMVDY

SEQ ID NO: 70 - protein, 60 aa, Epstein Barr virus
MVHVLERALLEQQSSACGLPGSSTETRPSHPCPEDPDVSRLRLLLAVLCVLFGLLCLLLI

SEQ ID NO: 71 - protein, 40 aa, Epstein Barr virus
MVHVLERALLEQQSSACGLPGSSTETRPSHPCPEDPDVSR

SEQ ID NO: 72 - protein, 96 aa, Bovine herpesvirus 1
MPRSPLIVAVVAAALFAIVRGRDPLLDAMRREGAMDFWSAGCYARGVPLSEPPQALVVFYVALTAVMVAVALYAYGLCFRLMGASGPNKKESRGRG

SEQ ID NO: 73 - protein, 54 aa, Bovine herpesvirus 1
MPRSPLIVAVVAAALFAIVRGRDPLLDAMRREGAMDFWSAGCYARGVPLSEPPQ

SEQ ID NO: 74 - protein, 199 aa, Human cytomegalovirus; identical to SEQ ID NO: 46

SEQ ID NO: 75 - protein, 161 aa, Human cytomegalovirus; identical to SEQ ID NO: 47

SEQ ID NO: 76 - protein, 38 aa, Human cytomegalovirus; identical to SEQ ID NO: 48

SEQ ID NO: 77 - protein, 186 aa, Human cytomegalovirus; identical to SEQ ID NO: 49

SEQ ID NO: 78 - protein, 160 aa, Human cytomegalovirus; identical to SEQ ID NO: 50

SEQ ID NO: 79 - protein, 26 aa, Human cytomegalovirus
TLLVYLFSLVVLVLLTVGVSARLRFI

SEQ ID NO: 80 - protein, 215 aa, Human cytomegalovirus; identical to SEQ ID NO: 52

SEQ ID NO: 81 - protein, 165 aa, Human cytomegalovirus; identical to SEQ ID NO: 53

SEQ ID NO: 82 - protein, 33 aa, Human cytomegalovirus; identical to SEQ ID NO: 54

SEQ ID NO: 83 - protein, 230 aa, Human cytomegalovirus
MERRRGTVPLGWVFFVLCLSASSSCAVDLGSKSSNSTCRLNVTELASIHPGETWTLHGMCISICYYENVTEDEIIGVAFTWQHNESVVDLWLYQNDTVIRNFSDITTNILQDGLKMRTVPVTKLYTSRMVTNLTVGRYDCLRCENGTTKIIERLYVRLGSLYPRPPGSGLAKHPSVSADEELSATLARDIVLVSAITLFFFLLALRIPQRLCQRLRIRLPHRYQRLRTED

SEQ ID NO: 84 - protein, 158 aa, Human cytomegalovirus
VDLGSKSSNSTCRLNVTELASIHPGETWTLHGMCISICYYENVTEDEIIGVAFTWQHNESVVDLWLYQNDTVIRNFSDITTNILQDGLKMRTVPVTKLYTSRMVTNLTVGRYDCLRCENGTTKIIERLYVRLGSLYPRPPGSGLAKHPSVSADEELSA

SEQ ID NO: 85 - protein, 46 aa, Human cytomegalovirus
TLARDIVLVSAITLFFFLLALRIPQRLCQRLRIRLPHRYQRLRTED

SEQ ID NO: 86 - protein, 338 aa, Human cytomegalovirus
MCRRESLRTLPWLFWVLLSCPRLLEYSSSSFPFATADIAEKMWAENYETTSPAPVLVAEGEQVTIPCTVMTHSWPMVSIRARFCRSHDGSDELILDAVKGHRLMNGLQYRLPYATWNFSQLHLGQIFSLTFNVSTDTAGMYECVLRNYSHGLIMQRFVILTQLETLSRPDEPCCTPALGRYSLGDQIWSPTPWRLRNHDCGMYRGFQRNYFYIGRADAEDCWKPACPDEEPDRCWTVIQRYRLPGDCYRSQPHPPKFLPVTPAPPADIDTGMSPWATRGIAAFLGFWSIFTVCFLCYLCYLQCCGRWCPTPGRGRRGGEGYRRLPTYDSYPGVKKMKR

SEQ ID NO: 87 - protein, 242 aa, Human cytomegalovirus
DIAEKMWAENYETTSPAPVLVAEGEQVTIPCTVMTHSWPMVSIRARFCRSHDGSDELILDAVKGHRLMNGLQYRLPYATWNFSQLHLGQIFSLTFNVSTDTAGMYECVLRNYSHGLIMQRFVILTQLETLSRPDEPCCTPALGRYSLGDQIWSPTPWRLRNHDCGMYRGFQRNYFYIGRADAEDCWKPACPDEEPDRCWTVIQRYRLPGDCYRSQPHPPKFLPVTPAPPADIDTGMSPWATR

SEQ ID NO: 88 - protein, 60 aa, Human cytomegalovirus
GIAAFLGFWSIFTVCFLCYLCYLQCCGRWCPTPGRGRRGGEGYRRLPTYDSYPGVKKMKR

SEQ ID NO: 89 - protein, 305 aa, Human cytomegalovirus
MRIEWACWLFGYFVSSVGSERSLSYRYHLESNSSANVVCNGNISVFVNGTLGVRYNITVGISSSLLIGHLTIQTLESWFTPWVQNKSYSKQPLSTTETLYNIDSENIHRVSQYFHTRWIKSLQENHTCDLTNSTPTYTYQANVNNTNYLTLTSSGWQDRLNYTAINSTHFNLTESNITSIHKYLNTTCIERLRNYTLEPVYTTAVPQNVTPEHAITTLYTTPPNAITIKDTTQSHTVQTPSFNDTHNVTEHTLNISYVLSQKTNNTTSPWVYAIPMGATATIGAGLYIGKHFTPVKFVYEVWRGQ

SEQ ID NO: 90 - protein, 251 aa, Human cytomegalovirus
ERSLSYRYHLESNSSANVVCNGNISVFVNGTLGVRYNITVGISSSLLIGHLTIQTLESWFTPWVQNKSYSKQPLSTTETLYNIDSENIHRVSQYFHTRWIKSLQENHTCDLTNSTPTYTYQANVNNTNYLTLTSSGWQDRLNYTAINSTHFNLTESNITSIHKYLNTTCIERLRNYTLEPVYTTAVPQNVTPEHAITTLYTTPPNAITIKDTTQSHTVQTPSFNDTHNVTEHTLNISYVLSQKTNNTTSPW

SEQ ID NO: 91 - protein, 35 aa, Human cytomegalovirus
VYAIPMGATATIGAGLYIGKHFTPVKFVYEVWRGQ

SEQ ID NO: 92 - protein, 205 aa, Human immunodeficiency virus
MGGKWSKSKTAGWPEVRERIRNAPSAAAPGVGAVSQDLAKHGAITSSNANHPSCVWLEAQEDEEVGFPVRPQVPLRPMTYKGALDLSHFLKEKGGLEGLIYSRRRQEILDLWVYHTQGYFPDWQNYTPGPGIRYPLTFGWCFKLVPVEPEEVEKATEGENNSLLHPICQHGMDDEEGEVLKWQFDPRLALKHRAQELHPEFYKDC

SEQ ID NO: 93 - protein, 81 aa, Human immunodeficiency virus
QPIPIVAIVALVVAIIIAIVVWSIVIIEYRKILRQRKIDRLIDRLIERAEDSGNESEGEISALVEMGVEMGHHAPWDVDDL

SEQ ID NO: 94 - protein, 333 aa, Human herpesvirus type 4
MEDEDVPVCWICNEELGNERFRACGCTGELENVHRSCLSTWLTISRNTACQICGVVYNTRVVWRPLREMTLLPRLTYQEGLELIVFIFIMTLGAAGLAAATWVWLYIVGGHDPEIDHVAAAAYYVFFVFYQLFVVFGLGAFFHMMRHVGRAYAAVNTRVEVFPYRPRPTSPECAVEEIELQEILPRGDNQDEEGPAGAAPGDQNGPAGAAPGDQDGPADGAPVHRDSEESVDEAAGYKEAGEPTHNDGRDDNVEPTAVGCDCNNLGAERYRATYCGGYVGAQSGDGAYSVSCHNKAGPSSLVDILPQGLPGGGYGSMGVIRKRSAVSSALMFH

SEQ ID NO: 95 - protein, 256 aa, Human herpesvirus type 4
MASKDVEEGVEGPICWICREEVGNEGIHPCACTGELDVVHPQCLSTWLTVSRNTACQMCRVIYRTRTQWRSRLNLWPEMERQEIFELFLLMSVVVAGLVGVALCTWTLLVILTAPAGTFSPGAVLGFLCFFGFYQIFIVFAFGGICRVSGTVRALYAANNTRVTVLPYRRPRRPTANEDNIELTVLVGPAGGTDEEPTDESSEGDVASGDKERDGSSGDEPDGGPNDRAGLRGTARTDLCAPTKKPVRKNHPKNNG

SEQ ID NO: 96 - protein, 201 aa, murine herpesvirus 68
MDSTGEFCWICHQPEGPLKRFCGCKGSCAVSHQDCLRGWLETSRRQTCALCGTPYSMKWKTKPLREWTWGEEEVLAAMEACLPLVLIPLAVLMIVMGTWLLVNHNGFLSPRMQVVLVVIVLLAMIVFSASASYVMVEGPGCLDTCTAKNSTVTVNSIDEAIATQQPTKTDLGLARETLSTRFRRGKCRSCCRLGCVRLCCV

SEQ ID NO: 97 - protein, 99 aa, Human T-cell lymphotropic virus type 1
MLFRLLSPLSPLALTALLLFLLPPSDVSGLLLRPPPAPCLLLFLPFQILSGLLFLLFLPLFFSLPLLLSPSLPITMRFPARWRFLPWKAPSQPAAAFLF

SEQ ID NO: 98 - protein, 245 aa, Cowpox virus
MKIKLSIIRWLTLLALTIFRMRSLVIVLLFPSIIYSMVIRRCEKMEEETWKLKIGMCIQAKDFYSKRTDCSVHRSDVGGGLITEGNGYRVVVHDQCEEPNPFIIATTKQTHFGVTHSYIEFSNSNTGAPENIPDCSKHILISVYCDQEASGLDFHTLKYVESNYLHITVKYDTSCINHLGVNYSFMNECERKLKSIYETDTLTCGAKDTQTRDKYLKTCTNTKFDRSVYKTHMQKSKILHVKTEL

SEQ ID NO: 99 - protein, 234 aa, Cowpox virus
MKIKLSIIRWLTLLALTIFRMRSLVIVLLFPSIIYSMVIRRCEKMEEETWKLKIGMCIQAKDFYSKRTDCSVHRSDVGGGLITEGNGYRVVVHDQCEEPNPFIIATTKQTHFGVTHSYIEFSNSNTGAPENIPDCSKHILISVYCDQEASGLDFHTLKYVESNYLHITVKYDTSCINHLGVNYSFMNECERKLKSIYETDTLTCGAKDTQTRDKYLKTCTNTKFDRSVYKTHMQ

SEQ ID NO: 100 - protein, 11 aa, Cowpox virus
KSKILHVKTEL

SEQ ID NO: 101 - protein, 245 aa, Cowpox virus
MKIKLSIIRWLTLLALTIFRMRSLIIFLLFPSIIYSMVIRRCEKMEEETWKLKIGMCIQAKDFYSKRTDCSVHRSDVGGGLITEGNGYRVVVHDQCEEPNPFIIATTKQTHFGVTHSYIEFSNSNTGAPENIPDCSKHILISVYCDQEASGLDFHTLKYVESNYLHITVKYDTSCINHLGVNYSFMNECERKLKSIYETDTLTCGAKDTQTRDKYLKTCTNTKFDRSVYKTHMRKSKILHVKTEL

SEQ ID NO: 102 - protein, 234 aa, Cowpox virus
MKIKLSIIRWLTLLALTIFRMRSLIIFLLFPSIIYSMVIRRCEKMEEETWKLKIGMCIQAKDFYSKRTDCSVHRSDVGGGLITEGNGYRVVVHDQCEEPNPFIIATTKQTHFGVTHSYIEFSNSNTGAPENIPDCSKHILISVYCDQEASGLDFHTLKYVESNYLHITVKYDTSCINHLGVNYSFMNECERKLKSIYETDTLTCGAKDTQTRDKYLKTCTNTKFDRSVYKTHMR

SEQ ID NO: 103 - protein, 11 aa, Cowpox virus
KSKILHVKTEL

SEQ ID NO: 104 - protein, 5 aa, synthetic construct
GGGGS

SEQ ID NO: 105 - protein, 8 aa, synthetic construct
GGGSGGGS

SEQ ID NO: 106 - protein, 15 aa, Homo sapiens
EPKSCDKTHTCPPCP

SEQ ID NO: 107 - protein, 12 aa, Homo sapiens
ESKYGPPCPSCP

SEQ ID NO: 108 - protein, 18 aa, synthetic construct
EGRGSLLTCGDVEENPGP

SEQ ID NO: 109 - protein, 21 aa, synthetic construct
GSGEGRGSLLTCGDVEENPGP

SEQ ID NO: 110 - protein, 19 aa, synthetic construct
ATNFSLLKQAGDVEENPGP

SEQ ID NO: 111 - protein, 22 aa, synthetic construct
GSGATNFSLLKQAGDVEENPGP

SEQ ID NO: 112 - protein, 20 aa, synthetic construct
QCTNYALLKLAGDVESNPGP

SEQ ID NO: 113 - protein, 23 aa, synthetic construct
GSGQCTNYALLKLAGDVESNPGP

SEQ ID NO: 114 - protein, 22 aa, synthetic construct
VKQTLNFDLLKLAGDVESNPGP

SEQ ID NO: 115 - protein, 25 aa, synthetic construct
GSGVKQTLNFDLLKLAGDVESNPGP

SEQ ID NO: 116 - protein, 274 aa, synthetic construct
MLLLVTSLLLCELPHPAFLLIPQIVLTQSPAIMSASPGEKVTMTCSATSSVSYMHWYQQKSGTSPKRWIYDTSKLASGVPARFSGSGSGTSYSLTISSMEAEDAATYYCQQWSSNPLTFGAGTKLELKGGGGSGGGGSGGGSEVQLQQSGPELVKPGASVKMSCKASGYKFTSYVMHWVKQKPGQGLEWIGYINPYNDVTKYNEKFKGKATLTSDKSSSTAYMELSSLTSEDSAVHYCARGSYYDYDGFVYWGQGTLVTVSAESKYGPPCPPCP

SEQ ID NO: 117 - protein, 789 aa, synthetic construct
MIHLGHILFLLLLPVAAAQTTPGERSSLPAFYPGTSGSCSGCGSLSLPLLAGLVAADAVASLLIVGAVFLCARPRRSPAQEDGKVYINMPGRGGGGSRVKFSRSADAPAYQQGQNQLYNELNLGRREEYDVLDKRRGRDPEMGGKPRRKNPQEGLYNELQKDKMAEAYSEIGMKGERRRGKGHDGLYQGLSTATKDTYDALHMQALPPRGSGEGRGSLLTCGDVEENPGPMGWIRGRRSRHSWEMSEFHNYNLDLKKSDFSTRWQKQRCPVVKSKCRENASPFFFCCFIAVAMGIRFIIMVTIWSAVFLNSLFNQEVQIPLTESYCGPCPKNWICYKNNCYQFFDESKNWYESQASCMSQNASLLKVYSKEDQDLLKLVKSYHWMGLVHIPTNGSWQWEDGSILSPNLLTIIEMQKGDCALYASSFKGYIENCSTPNTYICMQRTVGSGATNFSLLKQAGDVEENPGPMLLLVTSLLLCELPHPAFLLIPQIVLTQSPAIMSASPGEKVTMTCSATSSVSYMHWYQQKSGTSPKRWIYDTSKLASGVPARFSGSGSGTSYSLTISSMEAEDAATYYCQQWSSNPLTFGAGTKLELKGGGGSGGGGSGGGSEVQLQQSGPELVKPGASVKMSCKASGYKFTSYVMHWVKQKPGQGLEWIGYINPYNDVTKYNEKFKGKATLTSDKSSSTAYMELSSLTSEDSAVHYCARGSYYDYDGFVYWGQGTLVTVSAESKYGPPCPPCPGGGGSCLENTGTFCSTALLITALALVCTLLYLKYKSRRSFIDEKKMP

SEQ ID NO: 118 - DNA, 3212 bp, synthetic construct
  source 1..3212: mol_type = other DNA
atgctgctgctggtcacatctctgctgctgtgtgagctgccccatcccgcctttctgctgattccccagatcgtgctgacccagagccccgccatcatgtccgccagccccggcgagaaggtgaccatgacatgcagcgccaccagctccgtgtcctacatgcactggtaccagcagaagtccggcacctcccccaagaggtggatctacgacaccagcaagctggccagcggagtgcccgccagatttagcggcagcggaagcggaacatcctactctctgaccatcagcagcatggaggccgaggatgccgccacctattactgccagcagtggagcagcaaccctctgacctttggcgccggcaccaagctggaactgaaaggaggcggcggcagcggcggaggaggaagcggaggaggcagcgaggtgcagctccagcagtccggacccgagctggtcaagcccggagcttccgtcaagatgagctgcaaggccagcggctacaagttcaccagctacgtcatgcactgggtgaagcagaagcccggacaaggcctcgagtggatcggctatatcaacccctacaacgacgtgaccaagtacaacgagaagttcaagggcaaggccacactgacctccgacaagagctccagcacagcctacatggaactgagctctctgacaagcgaggattccgccgtgcactactgcgccagaggctcctactacgactacgacggctttgtgtactggggacaaggcacactggtcaccgtgagcgctgagagcaagtacggccccccttgccccccttgccccggcggaggcggaagctgtctggaatgattcatctgggccacattctgtttctgctgctgctgcccgtggccgccgctcaaacaacccccggcgagagaagctctctgcccgctttctatcccggcacctccggcagctgttccggctgtggatctctgtccctccctctgctggctggactggtggctgccgatgctgtggcctctctgctgattgtgggagccgtgtttctgtgcgccagacccagaagaagccccgcccaagaagacggcaaggtgtacatcaacatgcccggcagaggcggaggaggcagcagagtcaagttctctagaagcgctgatgcccccgcttaccagcaaggccagaaccagctgtacaacgaactgaatctgggaagaagagaggagtacgatgtgctggacaagaggagaggaagagaccccgagatgggcggcaaacctaggaggaagaaccctcaagagggactgtacaacgagctgcagaaggataagatggccgaggcctactccgagatcggaatgaagggcgagagaagaagaggcaaaggacacgatggactgtaccaaggactgagcaccgccacaaaggacacatacgacgctctgcacatgcaagctctgcctcccagaggaagcggcgaaggaagaggctctctgctgacatgcggagatgtggaagagaatcccggccccatggggtggattcgtggtcggaggtctcgacacagctgggagatgagtgaatttcataattataacttggatctgaagaagagtgatttttcaacacgatggcaaaagcaaagatgtccagtagtcaaaagcaaatgtagagaaaatgcatctccattttttttctgctgcttcatcgctgtagccatgggaatccgtttcattattatggtaacaatatggagtgctgtattcctaaactcattattcaaccaagaagttcaaattcccttgaccgaaagttactgtggcccatgtcctaaaaactggatatgttacaaaaataactgctaccaattttttgatgagagtaaaaactggtatgagagccaggcttcttgtatgtctcaaaatgccagccttctgaaagtatacagcaaagaggaccaggatttacttaaactggtgaagtcatatcattggatgggactagtacacattccaacaaatggatcttggcagtgggaagatggctccattctctcacccaacctactaacaataattgaaatgcagaagggagactgtgcactctatgcctcgagctttaaaggctatatagaaaactgttcaactccaaatacgtacatctgcatgcaaaggactgtgggaagcggcgctaccaatttctctctgctgaaacaagccggagacgtcgaggagaaccccggccccatgctgctgctggtcacatctctgctgctgtgtgagctgccccatcccgcctttctgctgattccccagatcgtgctgacccagagccccgccatcatgtccgccagccccggcgagaaggtgaccatgacatgcagcgccaccagctccgtgtcctacatgcactggtaccagcagaagtccggcacctcccccaagaggtggatctacgacaccagcaagctggccagcggagtgcccgccagatttagcggcagcggaagcggaacatcctactctctgaccatcagcagcatggaggccgaggatgccgccacctattactgccagcagtggagcagcaaccctctgacctttggcgccggcaccaagctggaactgaaaggaggcggcggcagcggcggaggaggaagcggaggaggcagcgaggtgcagctccagcagtccggacccgagctggtcaagcccggagcttccgtcaagatgagctgcaaggccagcggctacaagttcaccagctacgtcatgcactgggtgaagcagaagcccggacaaggcctcgagtggatcggctatatcaacccctacaacgacgtgaccaagtacaacgagaagttcaagggcaaggccacactgacctccgacaagagctccagcacagcctacatggaactgagctctctgacaagcgaggattccgccgtgcactactgcgccagaggctcctactacgactacgacggctttgtgtactggggacaaggcacactggtcaccgtgagcgctgagagcaagtacggccccccttgccccccttgccccggcggaggcggaagctgtctggagaataccggaacattctgctccacagctctgctgattaccgctctggctctggtgtgcacactgctgtatctgaagtacaagtctagaaggagcttcatcgatgagaagaagatgccc

SEQ ID NO: 119 - protein, 458 aa, synthetic construct
MLLLVTSLLLCELPHPAFLLIPDVVMTQTPLSLPVSLGDQASISCRSSQSLVHSNGNTYLHWYLQKPGQSPKLLIYKVSNRFSGVPDRFSGSGSGTDFTLKISRVEAEDLGVYFCSQNTHVPPTFGSGTKLEIKGGGGSGGGGSGGGGSQVQLQQSGAELVRPGASVKLSCKASGYTFTDYEMHWVKQTPVHGLKWIGALDPKTGDTAYSQKFKGKATLTADKSSSTAYMELRSLTSEDSAVYYCTRFYSYTYWGQGTLVTVSAESKYGPPCPPCPMFWVLVVVGGVLACYSLLVTVAFIIFWVKRGRKKLLYIFKQPFMRPVQTTQEEDGCSCRFPEEEEGGCELRVKFSRSADAPAYQQGQNQLYNELNLGRREEYDVLDKRRGRDPEMGGKPRRKNPQEGLYNELQKDKMAEAYSEIGMKGERRRGKGHDGLYQGLSTATKDTYDALHMQALPPR

SEQ ID NO: 120 - DNA, 1374 bp, synthetic construct
  source 1..1374: mol_type = other DNA
atgctgctgctggttacatctctgctgctgtgcgagctgccccatcctgcctttctgctgattcctgatgtggtcatgacacagacccctctgagcctgcctgtgtctctgggagatcaggccagcatcagctgcagatctagccagagcctggtgcacagcaacggcaacacatacctgcactggtatctgcagaagcccggacagagccccaagctgctgatctacaaggtgtccaaccggttcagcggcgtgcccgatagattttctggcagcggctctggcaccgacttcaccctgaagatctccagagtggaagccgaggacctgggcgtgtacttctgtagccagaacacccacgtgccacctacattcggcagcggcaccaagctggaaatcaagggaggcggaggatctggcggaggtggaagtggcggaggcggatctcaggtccagctgcagcagtctggagccgaacttgttagacctggcgcctctgtgaagctgagctgtaaagccagcggctacaccttcaccgactacgagatgcactgggtcaagcagacacctgtgcacggcctgaagtggattggagcactggaccctaagaccggcgataccgcctacagccagaagttcaagggcaaagccacactgaccgccgacaagagcagctccaccgcctatatggaactgcggagcctgaccagcgaggacagcgccgtgtactactgcacccggttctacagctacacctactggggacagggcaccctggttacagtttctgcagagagcaagtacggaccgccctgccccccttgccctatgttctgggtgctggtggtggtcggaggcgtgctggcctgctacagcctgctggtcaccgtggccttcatcatcttttgggtgaaacggggcagaaagaaactcctgtatatattcaaacaaccatttatgagaccagtacaaactactcaagaggaagatggctgtagctgccgatttccagaagaagaagaaggaggatgtgaactgcgggtgaagttcagcagaagcgccgacgcccctgcctaccagcagggccagaatcagctgtacaacgagctgaacctgggcagaagggaggagtacgacgtcctggataagcggagaggccgggaccctgagatgggcggcaagcctcggcggaagaacccccaggaaggcctgtataacgaactgcagaaagacaagatggccgaggcctacagcgagatcggcatgaagggcgagcggaggcggggcaagggccacgacggcctgtatcagggcctgtccaccgccaccaaggatacctacgacgccctgcacatgcaggccctgcccccaagg

SEQ ID NO: 121 - protein, 1268 aa, synthetic construct
MLLLVTSLLLCELPHPAFLLIPDVVMTQTPLSLPVSLGDQASISCRSSQSLVHSNGNTYLHWYLQKPGQSPKLLIYKVSNRFSGVPDRFSGSGSGTDFTLKISRVEAEDLGVYFCSQNTHVPPTFGSGTKLEIKGGGGSGGGGSGGGGSQVQLQQSGAELVRPGASVKLSCKASGYTFTDYEMHWVKQTPVHGLKWIGALDPKTGDTAYSQKFKGKATLTADKSSSTAYMELRSLTSEDSAVYYCTRFYSYTYWGQGTLVTVSAESKYGPPCPPCPMFWVLVVVGGVLACYSLLVTVAFIIFWVKRGRKKLLYIFKQPFMRPVQTTQEEDGCSCRFPEEEEGGCELRVKFSRSADAPAYQQGQNQLYNELNLGRREEYDVLDKRRGRDPEMGGKPRRKNPQEGLYNELQKDKMAEAYSEIGMKGERRRGKGHDGLYQGLSTATKDTYDALHMQALPPRGSGEGRGSLLTCGDVEENPGPMIHLGHILFLLLLPVAAAQTTPGERSSLPAFYPGTSGSCSGCGSLSLPLLAGLVAADAVASLLIVGAVFLCARPRRSPAQEDGKVYINMPGRGGGGSRVKFSRSADAPAYQQGQNQLYNELNLGRREEYDVLDKRRGRDPEMGGKPRRKNPQEGLYNELQKDKMAEAYSEIGMKGERRRGKGHDGLYQGLSTATKDTYDALHMQALPPRGSGEGRGSLLTCGDVEENPGPMGWIRGRRSRHSWEMSEFHNYNLDLKKSDFSTRWQKQRCPVVKSKCRENASPFFFCCFIAVAMGIRFIIMVTIWSAVFLNSLFNQEVQIPLTESYCGPCPKNWICYKNNCYQFFDESKNWYESQASCMSQNASLLKVYSKEDQDLLKLVKSYHWMGLVHIPTNGSWQWEDGSILSPNLLTIIEMQKGDCALYASSFKGYIENCSTPNTYICMQRTVGSGATNFSLLKQAGDVEENPGPMLLLVTSLLLCELPHPAFLLIPQIVLTQSPAIMSASPGEKVTMTCSATSSVSYMHWYQQKSGTSPKRWIYDTSKLASGVPARFSGSGSGTSYSLTISSMEAEDAATYYCQQWSSNPLTFGAGTKLELKGGGGSGGGGSGGGSEVQLQQSGPELVKPGASVKMSCKASGYKFTSYVMHWVKQKPGQGLEWIGYINPYNDVTKYNEKFKGKATLTSDKSSSTAYMELSSLTSEDSAVHYCARGSYYDYDGFVYWGQGTLVTVSAESKYGPPCPPCPGGGGSCLENTGTFCSTALLITALALVCTLLYLKYKSRRSFIDEKKMP

SEQ ID NO: 122 - DNA, 3804 bp, synthetic construct
  source 1..3804: mol_type = other DNA
atgctgctgctggttacatctctgctgctgtgcgagctgccccatcctgcctttctgctgattcctgatgtggtcatgacacagacccctctgagcctgcctgtgtctctgggagatcaggccagcatcagctgcagatctagccagagcctggtgcacagcaacggcaacacatacctgcactggtatctgcagaagcccggacagagccccaagctgctgatctacaaggtgtccaaccggttcagcggcgtgcccgatagattttctggcagcggctctggcaccgacttcaccctgaagatctccagagtggaagccgaggacctgggcgtgtacttctgtagccagaacacccacgtgccacctacattcggcagcggcaccaagctggaaatcaagggaggcggaggatctggcggaggtggaagtggcggaggcggatctcaggtccagctgcagcagtctggagccgaacttgttagacctggcgcctctgtgaagctgagctgtaaagccagcggctacaccttcaccgactacgagatgcactgggtcaagcagacacctgtgcacggcctgaagtggattggagcactggaccctaagaccggcgataccgcctacagccagaagttcaagggcaaagccacactgaccgccgacaagagcagctccaccgcctatatggaactgcggagcctgaccagcgaggacagcgccgtgtactactgcacccggttctacagctacacctactggggacagggcaccctggttacagtttctgcagagagcaagtacggaccgccctgccccccttgccctatgttctgggtgctggtggtggtcggaggcgtgctggcctgctacagcctgctggtcaccgtggccttcatcatcttttgggtgaaacggggcagaaagaaactcctgtatatattcaaacaaccatttatgagaccagtacaaactactcaagaggaagatggctgtagctgccgatttccagaagaagaagaaggaggatgtgaactgcgggtgaagttcagcagaagcgccgacgcccctgcctaccagcagggccagaatcagctgtacaacgagctgaacctgggcagaagggaggagtacgacgtcctggataagcggagaggccgggaccctgagatgggcggcaagcctcggcggaagaacccccaggaaggcctgtataacgaactgcagaaagacaagatggccgaggcctacagcgagatcggcatgaagggcgagcggaggcggggcaagggccacgacggcctgtatcagggcctgtccaccgccaccaaggatacctacgacgccctgcacatgcaggccctgcccccaaggggaagcggcgaaggaagaggctctctgctgacatgcggagatgtggaagagaatcccggccccatgattcatctgggccacattctgtttctgctgctgctgcccgtggccgccgctcaaacaacccccggcgagagaagctctctgcccgctttctatcccggcacctccggcagctgttccggctgtggatctctgtccctccctctgctggctggactggtggctgccgatgctgtggcctctctgctgattgtgggagccgtgtttctgtgcgccagacccagaagaagccccgcccaagaagacggcaaggtgtacatcaacatgcccggcagaggcggaggaggcagcagagtcaagttctctagaagcgctgatgcccccgcttaccagcaaggccagaaccagctgtacaacgaactgaatctgggaagaagagaggagtacgatgtgctggacaagaggagaggaagagaccccgagatgggcggcaaacctaggaggaagaaccctcaagagggactgtacaacgagctgcagaaggataagatggccgaggcctactccgagatcggaatgaagggcgagagaagaagaggcaaaggacacgatggactgtaccaaggactgagcaccgccacaaaggacacatacgacgctctgcacatgcaagctctgcctcccagaggaagcggcgaaggaagaggctctctgctgacatgcggagatgtggaagagaatcccggccccatggggtggattcgtggtcggaggtctcgacacagctgggagatgagtgaatttcataattataacttggatctgaagaagagtgatttttcaacacgatggcaaaagcaaagatgtccagtagtcaaaagcaaatgtagagaaaatgcatctccattttttttctgctgcttcatcgctgtagccatgggaatccgtttcattattatggtaacaatatggagtgctgtattcctaaactcattattcaaccaagaagttcaaattcccttgaccgaaagttactgtggcccatgtcctaaaaactggatatgttacaaaaataactgctaccaattttttgatgagagtaaaaactggtatgagagccaggcttcttgtatgtctcaaaatgccagccttctgaaagtatacagcaaagaggaccaggatttacttaaactggtgaagtcatatcattggatgggactagtacacattccaacaaatggatcttggcagtgggaagatggctccattctctcacccaacctactaacaataattgaaatgcagaagggagactgtgcactctatgcctcgagctttaaaggctatatagaaaactgttcaactccaaatacgtacatctgcatgcaaaggactgtgggaagcggcgctaccaatttctctctgctgaaacaagccggagacgtcgaggagaaccccggccccatgctgctgctggtcacatctctgctgctgtgtgagctgccccatcccgcctttctgctgattccccagatcgtgctgacccagagccccgccatcatgtccgccagccccggcgagaaggtgaccatgacatgcagcgccaccagctccgtgtcctacatgcactggtaccagcagaagtccggcacctcccccaagaggtggatctacgacaccagcaagctggccagcggagtgcccgccagatttagcggcagcggaagcggaacatcctactctctgaccatcagcagcatggaggccgaggatgccgccacctattactgccagcagtggagcagcaaccctctgacctttggcgccggcaccaagctggaactgaaaggaggcggcggcagcggcggaggaggaagcggaggaggcagcgaggtgcagctccagcagtccggacccgagctggtcaagcccggagcttccgtcaagatgagctgcaaggccagcggctacaagttcaccagctacgtcatgcactgggtgaagcagaagcccggacaaggcctcgagtggatcggctatatcaacccctacaacgacgtgaccaagtacaacgagaagttcaagggcaaggccacactgacctccgacaagagctccagcacagcctacatggaactgagctctctgacaagcgaggattccgccgtgcactactgcgccagaggctcctactacgactacgacggctttgtgtactggggacaaggcacactggtcaccgtgagcgctgagagcaagtacggccccccttgccccccttgccccggcggaggcggaagctgtctggagaataccggaacattctgctccacagctctgctgattaccgctctggctctggtgtgcacactgctgtatctgaagtacaagtctagaaggagcttcatcgatgagaagaagatgccc

SEQ ID NO: 123 - protein, 372 aa, synthetic construct
MAWRALHPLLLLLLLFPGSQAQSKAQVLQSVAGQTLTVRCQYPPTGSLYEKKGWCKEASALVCIRLVTSSKPRTMAWTSRFTIWDDPDAGFFTVTMTDLREEDSGHYWCRIYRPSDNSVSKSVRFYLVVSPASASTQTSWTPRDLVSSQTQTQSCVPPTAGARQAPESPSTIPVPSQPQNSTLRPGPAAPIAFWVLVVVGGVLACYSLLVTVAFIIFWVRSKRSRGGHSDYMNMTPRRPGPTRKHYQPYAPPRDFAAYRSRVKFSRSADAPAYQQGQNQLYNELNLGRREEYDVLDKRRGRDPEMGGKPRRKNPQEGLYNELQKDKMAEAYSEIGMKGERRRGKGHDGLYQGLSTATKDTYDALHMQALPPR

SEQ ID NO: 124 - DNA, 1116 bp, synthetic construct
  source 1..1116: mol_type = other DNA
atggcctggagagccctgcaccccctgctcctgctcctgctcctgttccccggcagccaagctcagtccaaggcccaagtgctgcagagcgtggccgggcagaccctgaccgtgagatgtcagtacccccccaccggcagcctgtacgagaagaagggctggtgcaaggaggcctccgccctggtgtgcatcagactggtgacaagcagcaagcctagaaccatggcctggacaagcagattcaccatctgggacgaccccgacgccggcttcttcaccgtgaccatgaccgacctgagagaggaggacagcggccactactggtgcagaatctacagacctagcgacaacagcgtgagcaagagcgtgagattctacctggtggtgagccccgcctccgcctccacacagacaagctggacccctagagacctggtgagcagccaaacacagacacagtcctgtgtgccccccaccgccggggctagacaagcccccgagagccctagcaccattcctgtccctagccaacctcagaattccaccctccggcccggccccgccgcccccatcgccttttgggtgctcgtggtcgtgggcggggtgctggcctgctacagcctgctggtgaccgtggccttcatcatcttctgggtgagaagcaagagaagcagaggcggccacagcgactacatgaacatgacccctagaagacccggccccacaagaaagcactatcagccctacgccccccctagagacttcgccgcctacagaagcagagtgaagttcagcagaagcgccgacgcccccgcctatcagcaagggcagaatcagctgtacaatgagctgaacctgggcagaagagaggagtacgacgtgctggacaagagaagaggcagagaccccgagatgggcggcaagcctagacggaagaacccccaagagggcctgtacaacgagctgcaaaaagacaagatggccgaggcctacagcgagatcggcatgaagggcgagagacggagaggcaagggccacgacggcctgtaccaaggcctgagcaccgccaccaaggacacctacgacgccctgcacatgcaagccctgccccctaga

SEQ ID NO: 125 - protein, 446 aa, synthetic construct
MIHLGHILFLLLLPVAAAQTTPGERSSLPAFYPGTSGSCSGCGSLSLPLLAGLVAADAVASLLIVGAVFLCARPRRSPAQEDGKVYINMPGRGGGGSRVKFSRSADAPAYQQGQNQLYNELNLGRREEYDVLDKRRGRDPEMGGKPRRKNPQEGLYNELQKDKMAEAYSEIGMKGERRRGKGHDGLYQGLSTATKDTYDALHMQALPPRGSGEGRGSLLTCGDVEENPGPMGWIRGRRSRHSWEMSEFHNYNLDLKKSDFSTRWQKQRCPVVKSKCRENASPFFFCCFIAVAMGIRFIIMVTIWSAVFLNSLFNQEVQIPLTESYCGPCPKNWICYKNNCYQFFDESKNWYESQASCMSQNASLLKVYSKEDQDLLKLVKSYHWMGLVHIPTNGSWQWEDGSILSPNLLTIIEMQKGDCALYASSFKGYIENCSTPNTYICMQRTV

SEQ ID NO: 126 - protein, 573 aa, synthetic construct
MLLLVTSLLLCELPHPAFLLIPQIVLTQSPAIMSASPGEKVTMTCSATSSVSYMHWYQQKSGTSPKRWIYDTSKLASGVPARFSGSGSGTSYSLTISSMEAEDAATYYCQQWSSNPLTFGAGTKLELKGGGGSGGGGSGGGSEVQLQQSGPELVKPGASVKMSCKASGYKFTSYVMHWVKQKPGQGLEWIGYINPYNDVTKYNEKFKGKATLTSDKSSSTAYMELSSLTSEDSAVHYCARGSYYDYDGFVYWGQGTLVTVSAESKYGPPCPPCPGGGGSCLENTGTFCSTALLITALALVCTLLYLKYKSRRSFIDEKKMPGSGATNFSLLKQAGDVEENPGPMERRRGTVPLGWVFFVLCLSASSSCAVDLGSKSSNSTCRLNVTELASIHPGETWTLHGMCISICYYENVTEDEIIGVAFTWQHNESVVDLWLYQNDTVIRNFSDITTNILQDGLKMRTVPVTKLYTSRMVTNLTVGRYDCLRCENGTTKIIERLYVRLGSLYPRPPGSGLAKHPSVSADEELSATLARDIVLVSAITLFFFLLALRIPQRLCQRLRIRLPHRYQRLRTED

SEQ ID NO: 127 - protein, 751 aa, synthetic construct
MLLLVTSLLLCELPHPAFLLIPQIVLTQSPAIMSASPGEKVTMTCSATSSVSYMHWYQQKSGTSPKRWIYDTSKLASGVPARFSGSGSGTSYSLTISSMEAEDAATYYCQQWSSNPLTFGAGTKLELKGGGGSGGGGSGGGSEVQLQQSGPELVKPGASVKMSCKASGYKFTSYVMHWVKQKPGQGLEWIGYINPYNDVTKYNEKFKGKATLTSDKSSSTAYMELSSLTSEDSAVHYCARGSYYDYDGFVYWGQGTLVTVSAESKYGPPCPPCPGGGGSCLENTGTFCSTALLITALALVCTLLYLKYKSRRSFIDEKKMPGSGATNFSLLKQAGDVEENPGPMERRRGTVPLGWVFFVLCLSASSSCAVDLGSKSSNSTCRLNVTELASIHPGETWTLHGMCISICYYENVTEDEIIGVAFTWQHNESVVDLWLYQNDTVIRNFSDITTNILQDGLKMRTVPVTKLYTSRMVTNLTVGRYDCLRCENGTTKIIERLYVRLGSLYPRPPGSGLAKHPSVSADEELSATLARDIVLVSAITLFFFLLALRIPQRLCQRLRIRLPHRYQRLRTEDGSGATNFSLLKQAGDVEENPGPMILGLLALAAVCSAAKKVEFKEPACNVTFKSEANECTTLIKCTTEHEKLIIRHKDKIGRYAVYAIWQPGDTNDYNVTVFQGENRKTFMYKFPFYEMCDITMYMSKQYKLWPPQKCLENTGTFCSTALLITALALVCTLLYLKYKSRRSFIDEKKMP

SEQ ID NO: 128 - protein, 438 aa, synthetic construct
MSSTLPALLCVGLCLSQRISAQQQTLPKPFIWAEPHFMVPKEKQVTICCQGNYGAVEYQLHFEGSLFAVDRPKPPERINKVKFYIPDMNSRMAGQYSCIYRVGELWSEPSNLLDLVVTEMYDTPTLSVHPGPEVISGEKVTFYCRLDTATSMFLLLKEGRSSHVQRGYGKVQAEFPLGPVTTAHRGTYRCFGSYNNHAWSFPSEPVKLLVTGDIENTSLAPEDPTFPADTWGTYLLTTETGLQKDHALWDHTAQNLLRFWVLVVVGGVLACYSLLVTVAFIIFWVRSKRSRGGHSDYMNMTPRRPGPTRKHYQPYAPPRDFAAYRSRVKFSRSADAPAYQQGQNQLYNELNLGRREEYDVLDKRRGRDPEMGGKPRRKNPQEGLYNELQKDKMAEAYSEIGMKGERRRGKGHDGLYQGLSTATKDTYDALHMQALPPR

SEQ ID NO: 129 - protein, 832 aa, synthetic construct
MAWRALHPLLLLLLLFPGSQAQSKAQVLQSVAGQTLTVRCQYPPTGSLYEKKGWCKEASALVCIRLVTSSKPRTMAWTSRFTIWDDPDAGFFTVTMTDLREEDSGHYWCRIYRPSDNSVSKSVRFYLVVSPASASTQTSWTPRDLVSSQTQTQSCVPPTAGARQAPESPSTIPVPSQPQNSTLRPGPAAPIAFWVLVVVGGVLACYSLLVTVAFIIFWVRSKRSRGGHSDYMNMTPRRPGPTRKHYQPYAPPRDFAAYRSRVKFSRSADAPAYQQGQNQLYNELNLGRREEYDVLDKRRGRDPEMGGKPRRKNPQEGLYNELQKDKMAEAYSEIGMKGERRRGKGHDGLYQGLSTATKDTYDALHMQALPPRGSGATNFSLLKQAGDVEENPGPMSSTLPALLCVGLCLSQRISAQQQTLPKPFIWAEPHFMVPKEKQVTICCQGNYGAVEYQLHFEGSLFAVDRPKPPERINKVKFYIPDMNSRMAGQYSCIYRVGELWSEPSNLLDLVVTEMYDTPTLSVHPGPEVISGEKVTFYCRLDTATSMFLLLKEGRSSHVQRGYGKVQAEFPLGPVTTAHRGTYRCFGSYNNHAWSFPSEPVKLLVTGDIENTSLAPEDPTFPADTWGTYLLTTETGLQKDHALWDHTAQNLLRFWVLVVVGGVLACYSLLVTVAFIIFWVRSKRSRGGHSDYMNMTPRRPGPTRKHYQPYAPPRDFAAYRSRVKFSRSADAPAYQQGQNQLYNELNLGRREEYDVLDKRRGRDPEMGGKPRRKNPQEGLYNELQKDKMAEAYSEIGMKGERRRGKGHDGLYQGLSTATKDTYDALHMQALPPR

SEQ ID NO: 130 - protein, 817 aa, synthetic construct
MSSTLPALLCVGLCLSQRISAQQQTLPKPFIWAEPHFMVPKEKQVTICCQGNYGAVEYQLHFEGSLFAVDRPKPPERINKVKFYIPDMNSRMAGQYSCIYRVGELWSEPSNLLDLVVTEMYDTPTLSVHPGPEVISGEKVTFYCRLDTATSMFLLLKEGRSSHVQRGYGKVQAEFPLGPVTTAHRGTYRCFGSYNNHAWSFPSEPVKLLVTGDIENTSLAPEDPTFPADTWGTYLLTTETGLQKDHALWDHTAQNLLRFWVLVVVGGVLACYSLLVTVAFIIFWVRSKRSRGGHSDYMNMTPRRPGPTRKHYQPYAPPRDFAAYRSRVKFSRSADAPAYQQGQNQLYNELNLGRREEYDVLDKRRGRDPEMGGKPRRKNPQEGLYNELQKDKMAEAYSEIGMKGERRRGKGHDGLYQGLSTATKDTYDALHMQALPPRGSGATNFSLLKQAGDVEENPGPMLLLVTSLLLCELPHPAFLLIPRKVCNGIGIGEFKDSLSINATNIKHFKNCTSISGDLHILPVAFRGDSFTHTPPLDPQELDILKTVKEITGFLLIQAWPENRTDLHAFENLEIIRGRTKQHGQFSLAVVSLNITSLGLRSLKEISDGDVIISGNKNLCYANTINWKKLFGTSGQKTKIISNRGENSCKATGQVCHALCSPEGCWGPEPRDCVSCRNVSRGRECVDKCNLLEGEPREFVENSECIQCHPECLPQAMNITCTGRGPDNCIQCAHYIDGPHCVKTCPAGVMGENNTLVWKYADAGHVCHLCHPNCTYGCTGPGLEGCPTNGPKIPSIATGMVGALLLLLVVALGIGLFM

SEQ ID NO: 131 - protein, 751 aa, synthetic construct
MAWRALHPLLLLLLLFPGSQAQSKAQVLQSVAGQTLTVRCQYPPTGSLYEKKGWCKEASALVCIRLVTSSKPRTMAWTSRFTIWDDPDAGFFTVTMTDLREEDSGHYWCRIYRPSDNSVSKSVRFYLVVSPASASTQTSWTPRDLVSSQTQTQSCVPPTAGARQAPESPSTIPVPSQPQNSTLRPGPAAPIAFWVLVVVGGVLACYSLLVTVAFIIFWVRSKRSRGGHSDYMNMTPRRPGPTRKHYQPYAPPRDFAAYRSRVKFSRSADAPAYQQGQNQLYNELNLGRREEYDVLDKRRGRDPEMGGKPRRKNPQEGLYNELQKDKMAEAYSEIGMKGERRRGKGHDGLYQGLSTATKDTYDALHMQALPPRGSGATNFSLLKQAGDVEENPGPMLLLVTSLLLCELPHPAFLLIPRKVCNGIGIGEFKDSLSINATNIKHFKNCTSISGDLHILPVAFRGDSFTHTPPLDPQELDILKTVKEITGFLLIQAWPENRTDLHAFENLEIIRGRTKQHGQFSLAVVSLNITSLGLRSLKEISDGDVIISGNKNLCYANTINWKKLFGTSGQKTKIISNRGENSCKATGQVCHALCSPEGCWGPEPRDCVSCRNVSRGRECVDKCNLLEGEPREFVENSECIQCHPECLPQAMNITCTGRGPDNCIQCAHYIDGPHCVKTCPAGVMGENNTLVWKYADAGHVCHLCHPNCTYGCTGPGLEGCPTNGPKIPSIATGMVGALLLLLVVALGIGLFM